European Patent Specification EP 3 500 685 B1, published July 12, 2023. Title: High Throughput Oil-Emulsion Synthesis of Bowtie Barcodes for Paired mRNA Capture and Sequencing from Individual Cells. Applicant: The Arizona Board of Regents on Behalf of Arizona State University. The sequence listing filed with the application follows.

SEQUENCE LISTING (2 sequences)

SEQ ID NO: 1 - DNA, 72 bp, Artificial Sequence
  Synthetic
cgagtccctttatcgggaacgaacgtggcgagaaaggaagggaacaaactatggacagcaaagacagcacct

SEQ ID NO: 2 - DNA, 111 bp, Artificial Sequence
  Synthetic
  misc_feature (50)..(61): n is a, c, g, or t
caccgactttgactcccaaatcaatgtgcggacagcaaagacagcacctnnnnnnnnnnnngctcagggaaatagcccttggggtagccttttgtttgtttgcaatctctg